European Patent Specification EP 3 523 319 B1, published June 28, 2023. Title: NUCLEIC ACID ENCODING SM1 RESISTANCE TO ORANGE WHEAT BLOSSOM MIDGE AND METHOD OF USE. Applicant: LIMAGRAIN EUROPE. The sequence listing filed with the application follows.

SEQUENCE LISTING (37 sequences)

SEQ ID NO: 1 - DNA, 8139 bp, Triticum aestivum
atgccggcagcagcggcggcgggtcaagttttccagtttccagtttcttagcagcggcaccatacggatcccacctgacaatatggccccacgatcaaataccacattgacttcatccacgtcagcaaaccacctttttttattttgacgggaaggtatactttattaggtcaaataacggttacgtcagcaaaccacctaagtgaacccatctaggaccatttctaaccggacgagatagataaggaggttaagagagcagaaaaaatgatcagggggttatgtgaaccatccattttgttcaggcttcgggggtggtattggtaaaatggacttttttttttcaggaaaaaaaaagaccaacgatctcctttttcctacacaaatctcccttctgcctcgtccaatgctcagctttcccttcttgctccgtcaaccgaactctccccctctccaacatttgtacccccaccagatcttgccccaaatctcttcttctccacaactcatgcccggaacctctcttccctgctccaaggcccaaagcttgcagcaaggcttcgcggttggaaatctgtgatggcttccccaaccccaactccaatctagatcttgctggtcttccccgagctcgtgttaccccgccggtgacggtcgtccgtgcggtactgagctccatcctctagcagtgcatctcggagtggcggtcacaccaaaagcataagttaatttgaggagcgagcgggtcaccgaggtatggaggtggtggtgggagtggcgagcgctgcggcgagcagcctggttccgaagctgctcacagtcttacagaacaagtggcgagggtcggaggacattgaagaggacgtctgctccttgcatcgagaggttgacatgatttatgcttctagcaaggatcagatctcgcacaaggggcagcccagtgaccaagagatcttgtctttgaaagaattctgtgatttggctcataacatcgaggactgcctagaccagttcattccttgcgctgaatgcggcaagggaaaactgaagatcctggatccaagcaagttccgtgatgagatcaagagactcaagcgggagctggatgcggcacaacagcggagggacagacacgtcgttgccgaatccaacgtcaacaacagcagcagcaccgctgtcgtggaggatacgggcaaaaaatatgaggcttgtcctgcagtgggcatcgagcaagcaaagggggagcttagggcgttgttagttggcggcgaagcaagcaagctgagggtggtctccatcctcggatttgggggctccggaaaaacagcactcgcctgggaagtgtacaaatgccctcaagtcgccaaggaattcagttgtcgtgcctgggcgaccatggcgtccgagcagaaacacgacatctctggcaaggaggcactcttgaaggctatacaaaaggggcttcttggagaaaaaacaccggagcccgtgcaacagacacccctggagctcgaaaacaatatcagtcatcttctccggattaataggtgaggattaatcctaaactgtcactcggaatattcacaacttgataccgtgaagaaatataagagcgtttagatcaccaaagtagtagtgatctaaacactcttatatttctttacagatatcttatcaccagtttagatctgcttaattgtaggattcagtttgtatctaagattcaaaggaatttgataggatttttggatgatttagatcattaggaatttctctatgcttgttgtttgattcatagttttggaatccttaggattcatttgtactctatttttggtggtacatttccatccgttgaaacctctttgtagatttcatttgttttttctgtgttgtaaaacacttttggtccaaatttcttcagttttataatcctatatgagattcaagaggacatggcactccaatcttgtcattttcttattcccgcattttgggaatcctaagattaacatgtgaccgaggtcttgcaagtgtccaagtacaagtatagttgtatcatcaggttttcactgacagtattaatatctcagttcaatatgaaacccaacgatcatagtgggtggcattgcccttaggctatttctggtgtcgttggtcactagttaattccagggggaaaatctgcacatggatttactaaaaaataaagaacttttcgtatttttagagttattcattagttatgcaaccagtaattgtaaaggctggaaaaaatggtaacgataagcaagaattttcgtccaaatactggacagattagctgatcaagtcattggttcgtatttccagtagaatgcttgcataccaaatatattctgaagatactttatcctctaatatagagttcagtagtctgaaacatttaccgatttggctgacaggtgtttaattgtaattgataacatcaagatggagctctggcacgcaataaaacctatcttcccagatgaaacggagagcagaatcctagtgaccacaactgtgacctcagtagctaatgcctgcagcttgcataacggttatgcgtacagtataagatctcttagtgcaaaacagtccaaggattatctagacaagaagcttttcgtcgatggatgctcattggatgtggagtggggtaccgcaatcgtgaacaaatgtgatggtcacccacttgctcttgttagtgttgccgaagctttgcaaggttgcggtgtggtgacaggagatcactgtgaagcaataagcgagaacctgggtttccgtatggaggagaactggaatggtcacttcacaaaactgcaacaagttctaatgaatgattacagcagtctgcctgacaattcttcaagaacctgcttactatacacaagtatattcccaaatagtcgccccttcaacacgaacagtcttacgaggcgattgtcagccgaagggtacatacagggtgatgataaacgcagtgcccagcaggttgcatatgaccacttggataaattgattgaccggaatatcatccggcctatcgacgcacacaacaattcaaaagtgaagacgtgcagaacacatggaatcatgaatcagttaatgttgtataagtccaggtcttcgaatttcatttctacatctattaatgataataaccgaagtaattaccgtcacctggttatccagaataacagaaacggtaaaagcttcagtccagaaacaagtgtcaagggcaagcagctgcgtccccggtctctaacagtctttgggagtgcagaagaagccgttccagatttgaagagttgtgagctgctgagagtgttggatctgaaagaatgcaatgatttgagggaccaacatctcgagcacatatacaagctgttgcatctaaaatatctggccctcggggattctagtagcaaatatctggatagaatgggaaagctacattgtttagagacactcgacttgaggaagaggaaaatcgagatactgccagtggaagtcatcagtttgccccacctagcacatctgttgggaaagttcaagctaaacaagttgggtaagaggaagcttaaagagttccggtcaaacaaatgcaacttggagactgtagcaggagttattgttgacagcgactctggattcctggaattgatggttcatttgaagcaacttagaaaggtcaagatatggtgcgagctcactagcacagattgcaagaacatactgggttcactttcaaaggccattcaaaagtttgctaaggatggcatagatactccagtaggtgaccgtggtcgcctatcactccatttcaacaattattctgaaggtctgttgcactgtgaagatgaccccacatttcttggttatcttaactcgctgaaactgcaaggcagcctgagtcagttccctaagtttgctaagtccctcgatggtctgcaagaactgtgccttacatatactaatctgacgggggctgatcttctactaggtctgtgtaggctacgacgcttggtttatctcaaactgatcgaagtccatcttgcggatttagacttagaagatggggatctcccaaaactgcaacgtctatgcctcgtggtgcaacagcccagattccccagtatccgaacaggcgctctgccgaaactaacttcaattcagttgctctgtggtggtctggaagatcttggtggcatcgaaatggaattgttcaaggacctccgggaaatcgctcttgattctacggtcaacccaaaaaccataaagctctgggaagatgaagctaagaagcaccccaagaggccaacggttatcttgctcgataaggttgttgctccagccgaagctacggcttcggtgaaatatgtcgcctcctgcaaagcctacaacaattgctacgccgacgctctggagcggaagttgcagaggtcatgtcaagtaacaccttcgcgcgagcaatccccgccacctcgctctcagcctgatcatcaagctcaagttcgcaatggattaggtttgcatatttctcatgccaatcattgctctgctaacatagcaaaataatgttgcatgtttagttgtcaataacgttctacacgttctggataactagaaatagtctcatttctattttgtgtattccagctttgccatcttgttttggagcaccagaagccggtgaagccgacggcgcacgtgatgctggactcgatccattgcatttgcattcgtcgtccgttgagcaggcgaacaagacagtgccatcgatcatgcccaacgggagcaaggaggtgtgagtgacacgggggcctggaaatctcttttctaggtcgtccagtctatttagtttctgaataaattccggccatgtaccagcattggcagatgcttctgtctggatgctgcatggcaaccgggaaaagacttactattttctattcatgtatcggtcaccttttaaatttcgtatttatgggttctgcaccccgaatctgtgttggaggataaatgtattatgtcagtcttatcaacgatttctcataaattcacttggatctgtttatttcgtgcgatttttttgtggtaggaatgcttttgttgaattttcttttgaaaaaaagcatgccgcaaaattcagaataggggaagggggtctttctgggcaagtccaagattatacgcaagaacagagcattttccctttttgcgggaagcgggaacagagcatgtgctctgctttgagcagagccggggccattctcctcctcttgggctcgactaaaaggttgtggcccagcccggcccgctcctcttgggttggaccaaaaggggcccgcccgactcatcggggagtatgcagcggcggcggcgcaggtgcttctccaagccgacccagtattttgagggtgaacggaatggtgattgcaagtccacgcatccgcaccgcgcgctagaatttgttagctggttaccccctcttccaccgaattgtagtgtaggcagcaatatatatatttgcttcccccgtggttagtatttttttttgaggataactttcaatttattcatcggctgtcaaagtagtacaaagaacaccagaagtaaaatatacatctagctaacagaaaagattagttttctgcatcaaattaatcagtatagttctcccccgtggtcaataggctgtcaattagcccatccaacttgcttctcgtggagcctcatgaagaggaaaagcgtgttttttttttctttcgcgttcaggcaaggatgtgcttccacaagagatgcttctcgaatgagaaaaaaaatcatgcttccgtccagggcctgccctgagggggtggcaggggggcggccgcccagggcccccgaaatctagggcccccctccagggttcgcaaggagcccatggcccaaaccataaggaggcgtcgacctagacgcacggagaaatccctgttttccttcttccccttgcgagttcgccgcttcgcgacgatcgtattcccccgagggccccggtcgcgagtcgcaacgccgatgtagatcgctctccgccatgcggccggctggtcttcctccaggtccccggtcccgtcgtgttatcccccgttcgtgagttttctctcatgtgcaagacgaaaccaccccacttataaagtcatccctaacctcctctttctagttggtcagatcttagaaggtctcgcatatgatgcagcagcagtcagcagtacaaaattgtagatggtgtttacaatagcccttttgttcatatggtgctaccgtacaaaatttacaattgtattgcatcatatcccccgcttgtctaattaagtaaaggaatacactatttacatttttcattttattttggaacaatagacaataataagttaggtaaaggaatgaatctaaaaagaaacgagattattattttgatctttatagtaggggccccgggttgtaatttcgccctggctcctgaaatatcaggaccggccctgcttccgtcttaggttttcttcttccggtttttttgtggaaaaaatttccatcgaaacctatgaacaagggatctagattcgaaaatctctatgggaaatcgaacggtgaaaacgcttcgcgatttagatgcacggtttaagagataaaccattttaaaatgatttatgtaaattgtttttgtaatatatttatttataatatttggaagtatagattgaagttaaaaaagaagtataaacgaggttgtggtctcccatgcgtctgggccggcccatctcgcgcgctgcttgatgtgaggcttccctcggtctcactacaagcaaggtatagctgcgctcgagcagaacccgcatcgcaacctatcggcttaccctcgcgggagctcctatctgccgctaactacggcaaatgtccaaggaacgcacaggcgggtctcccgactgggccgggccatgtggctctcccgttccggctagccaagaaactacatcgctcgctcgcaaaaaagaatgccctagcaggattcgaacacaataccacgtcgtgcttcacaagtattactcctaccacttgagctagcgagctaggtgttttcacggacagcgcaaatacttaagaaccaaaccaagcgcggatatgaacgtatttcaaatttcaacacgaaatattattttggagaaaaagtgaattctgtatgaaaccgcgaacacttttcgaaattgtgtatattttaaaaactcaaacatttcaaaaaacacaaacaatttctggaaactgaaacaatttttaaactccccccaagaaattgcaaaacattttgtacaaaactagaacattttttgaatggaaaaacaatttttagttacacaaacatttttgaaaaatgggaaaaaattgaatctcccgaaatttttttgagaacaccaacattttctgaaactcctgaacagagttcaatgcacaaactatttttaaaaattgcgaacaaattttgaaaacatgaacattacttaaaaaatcatgaacattttttatactcctgaacaaaaattgtaaacccaaatgctattgtaaatttgagacaattttcgtaatactgaacaaaatttgagaagttgcgaaatgctgaacaatttgtgataaatcaaacaatttttaaatttatgaacatttttccaataacataaaaaggaaaaacaaagaaaaaagaacacgaaaaaagagagaaaataataaacaaacaggaaaaaaagaaaaagaaaaaatgaaaagaaaaaacaggttcaggaacctactaagtcccaaaaccgggaacacccggctggaaccttccagcaaattattattagctagtgttggtggtgattagatagctaccgcagctagtgtttgttgtgattagctagctagaatgagtttaaaaatgatgatgtgctacactatgattatgatgattaaataactactgttggtggtaatgactatgatgatgattacatagcttgtgctggcggattagattcaagtggaggcaacatgtggtgcacatcaaaaatactactagtccaaactagatcaagtttggattag

SEQ ID NO: 2 - DNA, 4308 bp, Triticum aestivum
atgccggcagcagcggcggcgggtcaagaaaaaaaaagaccaacgatctcctttttcctacacaaatctcccttctgcctcgtccaatgctcagctttcccttcttgctccgtcaaccgaactctccccctctccaacatttgtacccccaccagatcttgccccaaatctcttcttctccacaactcatgcccggaacctctcttccctgctccaaggcccaaagcttgcagcaaggcttcgcggttggaaatctgtgatggcttccccaaccccaactccaatctagatcttgctggtcttccccgagctcgtgttaccccgccggtgacggtcgtccgtgcggtggtggtgggagtggcgagcgctgcggcgagcagcctggttccgaagctgctcacagtcttacagaacaagtggcgagggtcggaggacattgaagaggacgtctgctccttgcatcgagaggttgacatgatttatgcttctagcaaggatcagatctcgcacaaggggcagcccagtgaccaagagatcttgtctttgaaagaattctgtgatttggctcataacatcgaggactgcctagaccagttcattccttgcgctgaatgcggcaagggaaaactgaagatcctggatccaagcaagttccgtgatgagatcaagagactcaagcgggagctggatgcggcacaacagcggagggacagacacgtcgttgccgaatccaacgtcaacaacagcagcagcaccgctgtcgtggaggatacgggcaaaaaatatgaggcttgtcctgcagtgggcatcgagcaagcaaagggggagcttagggcgttgttagttggcggcgaagcaagcaagctgagggtggtctccatcctcggatttgggggctccggaaaaacagcactcgcctgggaagtgtacaaatgccctcaagtcgccaaggaattcagttgtcgtgcctgggcgaccatggcgtccgagcagaaacacgacatctctggcaaggaggcactcttgaaggctatacaaaaggggcttcttggagaaaaaacaccggagcccgtgcaacagacacccctggagctcgaaaacaatatcagtcatcttctccggattaataggtgtttaattgtaattgataacatcaagatggagctctggcacgcaataaaacctatcttcccagatgaaacggagagcagaatcctagtgaccacaactgtgacctcagtagctaatgcctgcagcttgcataacggttatgcgtacagtataagatctcttagtgcaaaacagtccaaggattatctagacaagaagcttttcgtcgatggatgctcattggatgtggagtggggtaccgcaatcgtgaacaaatgtgatggtcacccacttgctcttgttagtgttgccgaagctttgcaaggttgcggtgtggtgacaggagatcactgtgaagcaataagcgagaacctgggtttccgtatggaggagaactggaatggtcacttcacaaaactgcaacaagttctaatgaatgattacagcagtctgcctgacaattcttcaagaacctgcttactatacacaagtatattcccaaatagtcgccccttcaacacgaacagtcttacgaggcgattgtcagccgaagggtacatacagggtgatgataaacgcagtgcccagcaggttgcatatgaccacttggataaattgattgaccggaatatcatccggcctatcgacgcacacaacaattcaaaagtgaagacgtgcagaacacatggaatcatgaatcagttaatgttgtataagtccaggtcttcgaatttcatttctacatctattaatgataataaccgaagtaattaccgtcacctggttatccagaataacagaaacggtaaaagcttcagtccagaaacaagtgtcaagggcaagcagctgcgtccccggtctctaacagtctttgggagtgcagaagaagccgttccagatttgaagagttgtgagctgctgagagtgttggatctgaaagaatgcaatgatttgagggaccaacatctcgagcacatatacaagctgttgcatctaaaatatctggccctcggggattctagtagcaaatatctggatagaatgggaaagctacattgtttagagacactcgacttgaggaagaggaaaatcgagatactgccagtggaagtcatcagtttgccccacctagcacatctgttgggaaagttcaagctaaacaagttgggtaagaggaagcttaaagagttccggtcaaacaaatgcaacttggagactgtagcaggagttattgttgacagcgactctggattcctggaattgatggttcatttgaagcaacttagaaaggtcaagatatggtgcgagctcactagcacagattgcaagaacatactgggttcactttcaaaggccattcaaaagtttgctaaggatggcatagatactccagtaggtgaccgtggtcgcctatcactccatttcaacaattattctgaaggtctgttgcactgtgaagatgaccccacatttcttggttatcttaactcgctgaaactgcaaggcagcctgagtcagttccctaagtttgctaagtccctcgatggtctgcaagaactgtgccttacatatactaatctgacgggggctgatcttctactaggtctgtgtaggctacgacgcttggtttatctcaaactgatcgaagtccatcttgcggatttagacttagaagatggggatctcccaaaactgcaacgtctatgcctcgtggtgcaacagcccagattccccagtatccgaacaggcgctctgccgaaactaacttcaattcagttgctctgtggtggtctggaagatcttggtggcatcgaaatggaattgttcaaggacctccgggaaatcgctcttgattctacggtcaacccaaaaaccataaagctctgggaagatgaagctaagaagcaccccaagaggccaacggttatcttgctcgataaggttgttgctccagccgaagctacggcttcggtgaaatatgtcgcctcctgcaaagcctacaacaattgctacgccgacgctctggagcggaagttgcagaggtcatgtcaagtaacaccttcgcgcgagcaatccccgccacctcgctctcagcctgatcatcaagctcaagttcgcaatggattagctttgccatcttgttttggagcaccagaagccggtgaagccgacggcgcacgtgatgctggactcgatccattgcatttgcattcgtcgtccgttgagcaggcgaacaagacagtgccatcgatcatgcccaacgggagcaaggaggtgaatgcttttgttgaattttcttttgaaaaaaagcatgccgcaaaattcagaataggggaagggggtctttctgggcaagtccaagattatacgcaagaacagagcattttccctttttgcgggaagcgggaacagagcatgtgctctgctttgagcagagccggggccattctcctcctcttgggctcgactaaaaggttgtggcccagcccggcccgctcctcttgggttggaccaaaaggggcccgcccgactcatcggggagtatgcagcggcggcggcgcagggggtggcaggggggcggccgcccagggcccccgaaatctagggcccccctccagggttcgcaaggagcccatggcccaaaccataaggaggcgtcgacctagacgcacggagaaatccctgttttccttcttccccttgcgagttcgccgcttcgcgacgatcgtattcccccgagggccccggtcgcgagtcgcaacgccgatattgaagttaaaaaagaagtataaacgaggttgtggtctcccatgcgtctgggccggcccatctcgcgcgctgcttgatgtgaggcttccctcggtctcactacaagcaaggtatagctgcgctcgagcagaacccgcatcgcaacctatcggcttaccctcgcgggagctcctatctgccgctaactacggcaaatgtccaaggaacgcacaggcgggtctcccgactgggccgggccatgtggctctcccgttccggctagccaagaaactacatcgctcgctcgcaaaaaagaatgccctagcaggattcgaacacaataccacgtcgtgcttcacaacttgtgctggcggattagattcaagtggaggcaacatgtggtgcacatcaaaaatactactagtccaaactagatcaagtttggattag

SEQ ID NO: 3 - protein, 1435 aa, Triticum aestivum
MPAAAAAGQEKKRPTISFFLHKSPFCLVQCSAFPSCSVNRTLPLSNICTPTRSCPKSLLLHNSCPEPLFPAPRPKACSKASRLEICDGFPNPNSNLDLAGLPRARVTPPVTVVRAVVVGVASAAASSLVPKLLTVLQNKWRGSEDIEEDVCSLHREVDMIYASSKDQISHKGQPSDQEILSLKEFCDLAHNIEDCLDQFIPCAECGKGKLKILDPSKFRDEIKRLKRELDAAQQRRDRHVVAESNVNNSSSTAVVEDTGKKYEACPAVGIEQAKGELRALLVGGEASKLRVVSILGFGGSGKTALAWEVYKCPQVAKEFSCRAWATMASEQKHDISGKEALLKAIQKGLLGEKTPEPVQQTPLELENNISHLLRINRCLIVIDNIKMELWHAIKPIFPDETESRILVTTTVTSVANACSLHNGYAYSIRSLSAKQSKDYLDKKLFVDGCSLDVEWGTAIVNKCDGHPLALVSVAEALQGCGVVTGDHCEAISENLGFRMEENWNGHFTKLQQVLMNDYSSLPDNSSRTCLLYTSIFPNSRPFNTNSLTRRLSAEGYIQGDDKRSAQQVAYDHLDKLIDRNIIRPIDAHNNSKVKTCRTHGIMNQLMLYKSRSSNFISTSINDNNRSNYRHLVIQNNRNGKSFSPETSVKGKQLRPRSLTVFGSAEEAVPDLKSCELLRVLDLKECNDLRDQHLEHIYKLLHLKYLALGDSSSKYLDRMGKLHCLETLDLRKRKIEILPVEVISLPHLAHLLGKFKLNKLGKRKLKEFRSNKCNLETVAGVIVDSDSGFLELMVHLKQLRKVKIWCELTSTDCKNILGSLSKAIQKFAKDGIDTPVGDRGRLSLHFNNYSEGLLHCEDDPTFLGYLNSLKLQGSLSQFPKFAKSLDGLQELCLTYTNLTGADLLLGLCRLRRLVYLKLIEVHLADLDLEDGDLPKLQRLCLVVQQPRFPSIRTGALPKLTSIQLLCGGLEDLGGIEMELFKDLREIALDSTVNPKTIKLWEDEAKKHPKRPTVILLDKVVAPAEATASVKYVASCKAYNNCYADALERKLQRSCQVTPSREQSPPPRSQPDHQAQVRNGLALPSCFGAPEAGEADGARDAGLDPLHLHSSSVEQANKTVPSIMPNGSKEVNAFVEFSFEKKHAAKFRIGEGGLSGQVQDYTQEQSIFPFCGKREQSMCSALSRAGAILLLLGSTKRLWPSPARSSWVGPKGARPTHRGVCSGGGAGGGRGAAAQGPRNLGPPSRVRKEPMAQTIRRRRPRRTEKSLFSFFPLRVRRFATIVFPRGPRSRVATPILKLKKKYKRGCGLPCVWAGPSRALLDVRLPSVSLQARYSCARAEPASQPIGLPSRELLSAANYGKCPRNAQAGLPTGPGHVALPFRLAKKLHRSLAKKNALAGFEHNTTSCFTTCAGGLDSSGGNMWCTSKILLVQTRSSLD

SEQ ID NO: 4 - DNA, 10607 bp, Triticum aestivum
atgcggatgggcgggacacgcgcgcttgtccgtccctggcccgcatgtcagcgacacaaagtaaaacccctctgcggcccctttggcgccatcctccccccccaaaccctcccacatcccgcccgtcccactcccttccccgtccatggccgacgcccagccgaactcctgcgggctggccgtcgacccccccccccccgaatggccaagaagaagaaggacaaggcgccaaggaagccgcggtcggagtgcacgccggaggagatcgccaagttggacgcggaatcggtgaagaggaggggccggagggcggtcgccaaaaccaacatcgccgcggccaagagagttgccgagcgcgctgcgattgaggccgcacggcacaaggccgaggtcgaggagaaggaggccatcgtcagcaaagcgcgcgcccttctcatggctggcatttgtcgtccgcccggtttctctggaagggccgtcggtccggcgagcacaaggtcgtcggtcgcccggcctccgcactgccagtcgccgacatcgcggaccacgcccttgtcgcccggctttcctccaccaaggcacgacggccagacccgtttcggggggtcgccggatgtgagcatgatcgcgccgtccacaccacgcccctcggccgtcatcgacctcaacgtcacccttgggtccagcagcggcggccggccgtcggtcgagatgcaaagaaagcaagcacggctgccgtttaccggcaccatgccgtccccccgcgtcttgttcgatggaatgccaacaccaacgataccagtcgacgacccctagtatggccagttcatggaggaagtgatctacgagggttggcacgtccctgtctatgatcccgaggagacccaaagtcaggatggctgcggccagttcactgccgatgaagaggccaacgaccgtgctgactacgatcatggtgactcgtggcatgaagacgatgacatttatgtcgaaggtgatggtgatgaagaagaaagaaatgacgttgacattagtgttgagccattgttcatcgacgagctgacacaaagagcggaagcacaaaagaagaggaagagcattcgcacgagttcatacacacaagatgaggacaagttgatttgccaagcttggatggagattagccaagatccaaggaccggcgcgcaacaaaagggtattgttttttggacgagagtccacaaaacattccatgaaaggaagttgtttgagccctaccaatttgaaagcaaccgtggcatcggctcgattcaaaagagatggttgttcatccaacaagagtgcaacaagtatcaagccgcatttgagagcgttcaagcacggcccgtgagtggtctcggcgttggggacatggtatgctcttcttccttgccctttccttgctacggccatgagacttcggccttgtacatgtttgcatgttcacttgttgttgatcatatgttgtaggcatttcaatctttggaggcattcaaggcccggcacaatgacacgccgttcactcttacgcattgttggactatgatcaacatttgccctaagttcaaggaccaataccgtgaactccaaaggaagagaggcctgaagacggccaagtacgccggaggtggagatggcgaggcgttcaagaggccgaggggcaagaccaactccaaggttgacgacatacgtgatgcctcatccatggcattgcatgacactttgcatgacatgatgtcgcaaaaggatgtgaggaacgagaagaagcggcaaagcaatggcaagcaaatgaagcaatacctagagcttcaaacgaagaagcttgagatggaggaggcggctaagagaaggaagatcggcatggaggaggaggtccggcagaggcagctcgacatcgaggccatcaatgccgccaccaaagcgaaggaggtggccctcgcgatcatgagcgtggacttgtcgaagatgagtgagaagacgagggcctggttcgaggccaggcagaaggagatgctcgacgccgacggcctgaactaggtcgtccgatcggccgtggccgttcttttttggaggctggcatgggtaccgcgcgcccgctgggccgctggccatgtgccggcgagaaaaacatttattttgaaggtcggctgtgttgccggccgctggctgtgttgccgacgaggacgtccattcattttggaggctggctgtgttagcggccgctggcgtgatggacgtgtatgtcgctggctttgttgccggcgtgcgtgatgaactggggccgtagggcttggcatttgaaatgttgcttttttttaaatagacgcggacatggggctggacgcacggccaccgcatctcagaccaggcccggacacgaccccatctcctgaccaaacggacagaatccggacaaatcgaacatccgggtcgcgcggtggagttggccttaggcccgcgtaagaggcgttcaacgtactactaaacgtccacaaaaaaaaacgtactactaaacgtctaccagcggactcgacacctcgtatatgttgggcagtgcgaggagaacaaagaagacgttgacgcgttgacgctgctcaagggcgcagctgagggcgctgcagagttcaagcgcgcggcgcggcgcagatctctaccgtcgggcaggaggagaagcccgaggaaccaatgaagcctgagcccgacccgggcgtcgccgtctggcagcccgacggcgacgggtgaggatttttcgtgtttcctccctcctccgctccgggatttggccttcttgttagttactttggtgctcgctcttgtgtttctgttgcagagagatcgacatggatctgctgcctccgattagcgcgtctctgggcgccatggcctccctttccgggaagctggatgcgctccaggataccgaactcaaggatgagatccggaaacttggatcccggctgctgaagctctccgagccacatgaaccccgtcatgcggcgaggatctggatgaatgaggcgcgcgaactatcctatgacatggtaaactgtgtcgacgcggatgcagactggatcgacaagatgtcaagaatattcaagccacgcgtgaaggaggccaatgggcggtaccacagatacaagcttgagagcgtccccagccgtgcagctgtcttagcgatcccaatggtggtcggcgacgccggccggaagccagatctactcgtcggccttcacgccaatggtggcgccttcgaaacgctccgcaaaaatctgattgaccgggacgagcagctcaaggcgctattcgttgttggtgttggaggaatcggcaagaccacgcttgccaaagagctatggcgtgagcacaaacccgggcaccacttctgctgccgggctttcgtgcggaccgccaagaaacctgacatgaggaggatcctgaggagcatactcgcacaagttcgtccggatcaaccacccgtcgctaatgaggtgcacgagctcattcacgacctcaccgagcatctaaaggataaaaggtacttgagctgttgagcacctttcttctttaatatatatatatgatatgtacgctcttgcatattcaagaaaaaaatgtacttgagaaatgtatatagaactttcatcattctgataagactacttgaatagcgagtggtttttctacacccacgctagatgcagccatttcttaattcattataaggtgttttaatcttgaacaatgaagtattttctaaatccctgcaaacaaattattttctaagtgtttatattggtacaccattttcactcaaataaggttttggtgggtcttactgtcacaccaactgcaaacagaataacttgcctctgacaatagaaatgcactcagccaaaagacttacaaagttcattctgcaacatagcagtctaagtgtggaggagaaaattactagggtggagaagtgacaatctatagtctgcaccttgataaaaaaagtatatttcccacaaaataagagtagaaagtacaatatgcaaaaacggcattttcctcttgtgaaaacagagtggtcttcttgtgaaaacagagtctgtctactttgtggtgttgtcttcaatgccctagtgacacaacagtgcattgatttttctatgtgtttttccttctttgctgacttgtgtgtggatggtctcgtgatcttctgttcttgaccgtcccatcatcttgagcttgcgaggattggtgactcactagggcctagggtgtgccatggcgtgcctcctgagagggagatgtgcgtacttgtcttagcatcagtccaattagcactttcatgtcaaaccgagacttttctcgtgctacgtgtggtcggcacggcagggtcggagcagcggaggcgtgcgcagccatctctctcctaacgcgcggccggagaataaccacacacggaggctggtcgtctcggccggcgcgccgttgcggagaaggagtggacctccgtctctcgcggcccgggccgaagcctcgacgacggagcggatgtgctgcggtcgcggtccgggagcgccatcgccgctcgatctgggtagcaagagaaggtgagggcgcggcggcgtggggagaagaaggcggagggagacggcgtcgccggtgggagagaaggtgaggggagcggcggcgtttgcagacgaggtcgccggtgggagagaaggtgaggggagcggcggcggcggtgttgagtcgggagaggaggagagcgggcgagggttgggtttgtgttcgttttttctttttttttcctttttgtgagctgggctcggtgaattatctccctccctccctctctcctttttttctctttttcattttgaaatctagtagcgggagcaattaaggcctcaacattatttcgaggcgactaaaataaatattttggcgggagctttcaggttgattggttgggcagcgcaccgtctcaaaattcaaggacgcccttgatatatgatccgaaattcatggctattagaaaactaaaaacaaattagcagttaactgaccttttgattggctattcgtgctacgtggcataagccagcgggcgcccagcgtttcgttgataatgggtttgatggtttcagagctgatacccatgatgacactcctaattagttgcactcagcaatctgtgaagcaacaataagccagttaataggatgttggacaatctcttttccttctttattccatggcacgtatccattaattttgccttttatttgcatgaaagtgttatgggtatgcaagggtggcactgacctgatgtgtaaggttaggtactcgaacttatgagtgtagcactgaaataactgtgtgcttgttttaggagtatttgtggtattccatttacatttaattatactatatactttgtttatcaggtacttcattataattgatgacttatgggatacatcagtatgggatgttgcagcccgtgctttcccaaagggtaaccaaggcagcaggatagtaacaacaacggaaattgaggatgttgctcttgcatgttgttatcagtcaaagtacgtgcttaagatggaacatcttagcgagagtcactcaagagagttgttcaccagtgcagtgtttcgctctggagaacaacactctcaccacgtaggtgaagtgccagatgagattataagaagatgtgctggtttaccacaggcaattatcagcatatccagtgttctagcaagccatggagaagcaaatacagtaaagaactgggagcaaatacaaaacagtttgccaacaaatacaacttctgacgagatactgaaagaagtactgattttttgctataatagtcttcccagttgtgttcagacatgtctgttgcatcttagtatatacccggagaactatgttatcttgaaggaagatataacgaagcaatgggttgctgaaggtctcatcagtgcaccaacagagaaagaaaaaatggaaattgccaggagctattttgatatgcttgtcagtatgggcatgatccaacatatagacgtagactatggcaatgatgttttgtactatgcggtgcatcacatggtacatgatatcattacatccaagtccatagaagagaattttgttaaagtaatagattattctcaaagggcggtacggttttctaacaaggttagtcgtctgtccctccagtttggcggtgcaacatatgcaactacaccagcacgtatcgaactgtcgcaagtgcgatctcttgcttatactggactgaagagctgcttgccttccatctcagagtttaagcttctccgggtactgattctccatatttgggctgatcaaccaagcacatgtgtcactcgcaaaaaaaagaaccaagcacaggtgtccacctcgagtgtatctctcgattgcttctattaatatatttgcaggtgacatgcaacggcaccgtgcatcttccaaaacagatgcgatgtctgaaacacttggaaacacttgaaataaatgcaacagtagcagccattccatcggatattgttcatcttcggagcttgttgcatctccgtctaggaggtgggacagaactgcctgatgtgacaggtgtcctcacaaatgttaccctgaatcttcctagtgctgccactttattggatgattcgagcagttctcccgattcactgaacacaatggagctattgccacccatttgcagaatccccaactggattggacagcttactgacctctgcattctgaaagttgtcgtcagagaactgctaagggatgatatcagtaacctggaaagattgccagcactcactgttctctccttgtacgtccagcaaagaaatacagaactaatcattttcgaagccggagcattttctgctctcgagtgttttgagttcaggtgtggtgaactgcagctgatgtttcaggaaggagcaatgcccaatcttcacagaatcaagctaggtttcaatgctcacaaaggagaacagtatgatcgtcttcttagcggcattgagaacctgtctgacgtccaggaaatttctggaataattggggcagcccctggtgccgatgagcatgactttcaggctgcagaatctgcattcatgaaagctgttagcaagctctctagtaaagtcagtgtaaaaagagcagatatggttgaggaagagggtggcctggcagaaaaacaggatgtgatccgagagaaagatgcatcaagacatgtaataagtgaacagcctgcaattctgaaacaagagtctgaggaagatataaagcaaaatgctggtggcagtttgcctagcggcattaagaacctgtcaaacgtccaggaaatttctggaataactggggtagccacaggtgctgaggaacatgaaattcaggctgcagaatctgcattgatgaaatccgtcagtgagcaacctagtaaggtcactataaaaggagcagatatggttgagcaagggtatggtccggcagacaaacaacatgtgagccgagagaaagatgtatcaagccatttaagaagtgaacaacctgcaattgtgaaacaagagtccggtggcaactctcagttcattcaatggtacggttctttgtcctgttatgtccattatttcacactttctctttctttggtgaacttccattacactcttctgcctcacacagtaatagctaaacataggtcatcaccaactttgaactttattttgcactgacgttgcactcttttaaatgggtgtgatttgtgcaaagctccattgctcaagtaacagaggtcaaggagaagaacgaataaattggtcatatatgtttaaagcttgctctagatgtaaaaatatatccataaaatttcgcaaatgtggaacatccttattttcttagcaggagaagcaatagcaaggaaacttcaaacgtggtgcaaggtttgtcagggaaccgagaacttcgtggcggtgctgttggagaagttaacaaggtatggttttgttttgtaagggaacatggtacgatttaagacatacatagtacttacatacttctgaaaccatcgctcaagtcccatgatttcaaatgtgcatgattatctaacaccatatttgatcatgttttttgcaagttttacttcttggatatatgcacagatgtgacaatccaaatgtactagtagtacataactttgaaaatatcagccaaattcagtgatttcagggtattagatcacatacactgaaatcagtgtatgctgcatacctaaattcaggacaggttatccaaaactaacccaaaattctttttaactttttgtgatttttttcatacgtatgtggtacattttgatttttatgactaggtaaagaaactaatgttgacaaaaagccaggcttgcttttaatttccgtatttgatttttaaatcatggagctagctatcatagattccacatttaccagggagctagctggagagccaaaaagtggattaagaatgatcattgtggatgttgaacatattctctcctcttaggtgaaatatttttctctctttctcaggaagaagaacgtcagaatagcctggcgagaggcaaaagcagcatggatattaaactcgtggagatcgaagccatcacaaacaattttgcagaggaacagaaagtcggcagcggtgggtacggagatgtttacagggtatgttcttttactactgatcattgtattttctgtctgtatttctcacatttacaatcaagatctgtactatgacaagtcgtcgattttatcaggccactcacaaaggagaggaagttgccgtgaagaagctccatcaactgcagggactcgatgataagcaattcgacagcgagttccgtaaccttcgtaatatacgccaccaaaatgttgtgcggctaattggctactgccacgagtctcgcaagaaatacatggagcacaagggggagctcatcttcgccaaagagatggagcgcgtgctctgcttcgaatatatgcacggcggaagcctcgataaacatattacaggtcattaactctcttctgtgacctgcatccaagatatatgaatgattcagcatcatatatctgacaaatacgctgctgtgtttacttgtaattgcagatgaatcttgtgagcttgattggccgacgtgttacaaaatcatcaaagggacttgtgagggcttaaatcaccttcacacctcgcaggggaagcctattttacatctagacataaaaccagccaacatattgctggataagagcatgacgcctaaaatcgccgatcttggtttgtccaaacttgtttcttcgacattaacacataaaacagagattgtcaaagggacacagtaagttgatgcatagtttaggcttgcttcgttcttgtatgacttgaaactgagcctttgtttctcttgcaataaccatatctattatgcttttgatgatatcttgcagagggtacatgccgccagagtatgtagacaatggccagatatcgaacaagtttgacgtgtttagttttggcgtagtaattataaaaatgatggccggtaacgtgggctacttccgttgtgctgaaatgtctcacaaagagtttattgagctggtaagaaaaataccccctgttgattccatgaatatataattatacatacatctcagcctctctctttttgggggtgtctcttccaagtgttagtatactctaggaagctttatgcgccaactttgcatgtaggtaactaaaaactgggtgaaaaggttgctgacagagcctggatattcctcgcacgaaaccgacatgctaggagtcactagatgtgttgaaattgcattaagatgtgtggacaaggaccgaaacaaaaggccctgtattaaggatgttgtccatgagctggaggaactagaagctgagatcaagaaaatgtccctatcttccgaccagtcaaaaggcctaagtctgcaggcaagcatccttgtcactctttgtactaggttttgcaactctctgttttttcacagtagcattcagccctgacaaacttctgtcaaatttgtatcaacgtagcgatgtttgtacgaccggatgcagtaactgacgccttattttcttttcagagaagctgtgacaccaacattctctcggtggatccgaccctcgagctgcggttcgtctttgagccaaggaaggagacgtcgtgctgtctgcagatgaccaacaagacgggtggcttcatcgcattcaacatattgatgaacaagaacaagtatagtgtgcggccaagccaagggaccatgccaccgtgctccaggcgttatgttgtcgtgacactgtcagcgcaagaggcggcgccgccatacatgcggtgtgacgacatgctcctagtgcagagcaccagcatcacccaagatcttggtgagatcaattatcaagaattgttcgacgtggccagggcggataaggtggttgatgtggtgcatctgccaatcgcatatgtcacgttagaagagtag

SEQ ID NO: 5 - DNA, 6912 bp, Triticum aestivum
atgcggatgggcgggacacgcgcgcttgtccgtccctggcccgcatgtcagcgacacaaagtaaaacccctctgcggcccctttggcgccatcctccccccccaaaccctcccacatcccgcccgtcccactcccttccccgtccatggccgacgcccagccgaactcctgcgggctggccgtcgacccccccccccccgaatggccaagaagaagaaggacaaggcgccaaggaagccgcggtcggagtgcacgccggaggagatcgccaagttggacgcggaatcggtgaagaggaggggccggagggcggtcgccaaaaccaacatcgccgcggccaagagagttgccgagcgcgctgcgattgaggccgcacggcacaaggccgaggtcgaggagaaggaggccatcgtcagcaaagcgcgcgcccttctcatggctggcatttgtcgtccgcccggtttctctggaagggccgtcggtccggcgagcacaaggtcgtcggtcgcccggcctccgcactgccagtcgccgacatcgcggaccacgcccttgtcgcccggctttcctccaccaaggcacgacggccagacccgtttcggggggtcgccggatgtgagcatgatcgcgccgtccacaccacgcccctcggccgtcatcgacctcaacgtcacccttgggtccagcagcggcggccggccgtcggtcgagatgcaaagaaagcaagcacggctgccgtttaccggcaccatgccgtccccccgcgtcttgttcgatggaatgccaacaccaacgataccagtcgacgacccctatcaggatggctgcggccagttcactgccgatgaagaggccaacgaccgtgctgactacgatcatggtgactcgtggcatgaagacgatgacatttatgtcgaaggtgatggtgatgaagaagaaagaaatgacgttgacattagtgttgagccattgttcatcgacgagctgacacaaagagcggaagcacaaaagaagaggaagagcattcgcacgagttcatacacacaagatgaggacaagttgatttgccaagcttggatggagattagccaagatccaaggaccggcgcgcaacaaaagggtattgttttttggacgagagtccacaaaacattccatgaaaggaagttgtttgagccctaccaatttgaaagcaaccgtggcatcggctcgattcaaaagagatggttgttcatccaacaagagtgcaacaagtatcaagccgcatttgagagcgttcaagcacggcccgtgagtggtctcggcgttggggacatggcatttcaatctttggaggcattcaaggcccggcacaatgacacgccgttcactcttacgcattgttggactatgatcaacatttgccctaagttcaaggaccaataccgtgaactccaaaggaagagaggcctgaagacggccaagtacgccggaggtggagatggcgaggcgttcaagaggccgaggggcaagaccaactccaaggttgacgacatacgtgatgcctcatccatggcattgcatgacactttgcatgacatgatgtcgcaaaaggatgtgaggaacgagaagaagcggcaaagcaatggcaagcaaatgaagcaatacctagagcttcaaacgaagaagcttgagatggaggaggcggctaagagaaggaagatcggcatggaggaggaggtccggcagaggcagctcgacatcgaggccatcaatgccgccaccaaagcgaaggaggtggccctcgcgatcatgagcgtggacttgtcgaagatgagtgagaagacgagggcctggctggcatgggtaccgcgcgcccgctgggccgctggccatgtgccggcgagaaaaacatttattttgaaggtcggctgtgttgccggccgctggctgtgttgccgacgaggacgtccattcattttggaggctggctgtgttagcggccgctggcgtgatggacgtgtatgtcgctggctttgttgccggcacgcggacatggggctggacgcacggccaccgcatctcagaccaggcccggacacgaccccatctcctgaccaaacggacagaatccggacaaatcgaacatccgggtcgcgcggtggagttggccttaggcccgcagttcaagcgcgcggcgcggcgcagatctctaccgtcgggcaggaggagaagcccgaggaaccaatgaagcctgagcccgacccgggcgtcgccgtctggcagcccgacggcgacggagagatcgacatggatctgctgcctccgattagcgcgtctctgggcgccatggcctccctttccgggaagctggatgcgctccaggataccgaactcaaggatgagatccggaaacttggatcccggctgctgaagctctccgagccacatgaaccccgtcatgcggcgaggatctggatgaatgaggcgcgcgaactatcctatgacatggtaaactgtgtcgacgcggatgcagactggatcgacaagatgtcaagaatattcaagccacgcgtgaaggaggccaatgggcggtaccacagatacaagcttgagagcgtccccagccgtgcagctgtcttagcgatcccaatggtggtcggcgacgccggccggaagccagatctactcgtcggccttcacgccaatggtggcgccttcgaaacgctccgcaaaaatctgattgaccgggacgagcagctcaaggcgctattcgttgttggtgttggaggaatcggcaagaccacgcttgccaaagagctatggcgtgagcacaaacccgggcaccacttctgctgccgggctttcgtgcggaccgccaagaaacctgacatgaggaggatcctgaggagcatactcgcacaagttcgtccggatcaaccacccgtcgctaatgaggtgcacgagctcattcacgacctcaccgagcatctaaaggataaaagggtcggagcagcggaggcgtgcgcagccatctctctcctaacgcgcggccggagaataaccacacacggaggctggtcgtctcggccggcgcgccgttgcggagaaggagtggacctccgtctctcgcggcccgggccgaagcctcgacgacggagcggatgtgctgcggtcgcggtccgggagcgccatcgccgctcgatctgggtagcaagagaaggtgagggcgcggcggcgtggggagaagaaggcggagggagacggcgtcgccggtgggagagaaggtacttcattataattgatgacttatgggatacatcagtatgggatgttgcagcccgtgctttcccaaagggtaaccaaggcagcaggatagtaacaacaacggaaattgaggatgttgctcttgcatgttgttatcagtcaaagtacgtgcttaagatggaacatcttagcgagagtcactcaagagagttgttcaccagtgcagtgtttcgctctggagaacaacactctcaccacgtaggtgaagtgccagatgagattataagaagatgtgctggtttaccacaggcaattatcagcatatccagtgttctagcaagccatggagaagcaaatacagtaaagaactgggagcaaatacaaaacagtttgccaacaaatacaacttctgacgagatactgaaagaagtactgattttttgctataatagtcttcccagttgtgttcagacatgtctgttgcatcttagtatatacccggagaactatgttatcttgaaggaagatataacgaagcaatgggttgctgaaggtctcatcagtgcaccaacagagaaagaaaaaatggaaattgccaggagctattttgatatgcttgtcagtatgggcatgatccaacatatagacgtagactatggcaatgatgttttgtactatgcggtgcatcacatggtacatgatatcattacatccaagtccatagaagagaattttgttaaagtaatagattattctcaaagggcggtacggttttctaacaaggttagtcgtctgtccctccagtttggcggtgcaacatatgcaactacaccagcacgtatcgaactgtcgcaagtgcgatctcttgcttatactggactgaagagctgcttgccttccatctcagagtttaagcttctccgggtactgattctccatatttgggctgatcaaccaagcacatgtgtcactcgcaaaaaaaagaaccaagcacaggtgacatgcaacggcaccgtgcatcttccaaaacagatgcgatgtctgaaacacttggaaacacttgaaataaatgcaacagtagcagccattccatcggatattgttcatcttcggagcttgttgcatctccgtctaggaggtgggacagaactgcctgatgtgacaggtgtcctcacaaatgttaccctgaatcttcctagtgctgccactttattggatgattcgagcagttctcccgattcactgaacacaatggagctattgccacccatttgcagaatccccaactggattggacagcttactgacctctgcattctgaaagttgtcgtcagagaactgctaagggatgatatcagtaacctggaaagattgccagcactcactgttctctccttgtacgtccagcaaagaaatacagaactaatcattttcgaagccggagcattttctgctctcgagtgttttgagttcaggtgtggtgaactgcagctgatgtttcaggaaggagcaatgcccaatcttcacagaatcaagctaggtttcaatgctcacaaaggagaacagtatgatcgtcttcttagcggcattgagaacctgtctgacgtccaggaaatttctggaataattggggcagcccctggtgccgatgagcatgactttcaggctgcagaatctgcattcatgaaagctgttagcaagctctctagtaaagtcagtgtaaaaagagcagatatggttgaggaagagggtggcctggcagaaaaacaggatgtgatccgagagaaagatgcatcaagacatgtaataagtgaacagcctgcaattctgaaacaagagtctgaggaagatataaagcaaaatgctggtggcagtttgcctagcggcattaagaacctgtcaaacgtccaggaaatttctggaataactggggtagccacaggtgctgaggaacatgaaattcaggctgcagaatctgcattgatgaaatccgtcagtgagcaacctagtaaggtcactataaaaggagcagatatggttgagcaagggtatggtccggcagacaaacaacatgtgagccgagagaaagatgtatcaagccatttaagaagtgaacaacctgcaattgtgaaacaagagtccggtggcaactctcagttcattcaatggagaagcaatagcaaggaaacttcaaacgtggtgcaaggtttgtcagggaaccgagaacttcgtggcggtgctgttggagaagttaacaaggaagaagaacgtcagaatagcctggcgagaggcaaaagcagcatggatattaaactcgtggagatcgaagccatcacaaacaattttgcagaggaacagaaagtcggcagcggtgggtacggagatgtttacagggccactcacaaaggagaggaagttgccgtgaagaagctccatcaactgcagggactcgatgataagcaattcgacagcgagttccgtaaccttcgtaatatacgccaccaaaatgttgtgcggctaattggctactgccacgagtctcgcaagaaatacatggagcacaagggggagctcatcttcgccaaagagatggagcgcgtgctctgcttcgaatatatgcacggcggaagcctcgataaacatattacagatgaatcttgtgagcttgattggccgacgtgttacaaaatcatcaaagggacttgtgagggcttaaatcaccttcacacctcgcaggggaagcctattttacatctagacataaaaccagccaacatattgctggataagagcatgacgcctaaaatcgccgatcttggtttgtccaaacttgtttcttcgacattaacacataaaacagagattgtcaaagggacacaagggtacatgccgccagagtatgtagacaatggccagatatcgaacaagtttgacgtgtttagttttggcgtagtaattataaaaatgatggccggtaacgtgggctacttccgttgtgctgaaatgtctcacaaagagtttattgagctggtaactaaaaactgggtgaaaaggttgctgacagagcctggatattcctcgcacgaaaccgacatgctaggagtcactagatgtgttgaaattgcattaagatgtgtggacaaggaccgaaacaaaaggccctgtattaaggatgttgtccatgagctggaggaactagaagctgagatcaagaaaatgtccctatcttccgaccagtcaaaaggcctaagtctgcaggcaagcatccttagaagctgtgacaccaacattctctcggtggatccgaccctcgagctgcggttcgtctttgagccaaggaaggagacgtcgtgctgtctgcagatgaccaacaagacgggtggcttcatcgcattcaacatattgatgaacaagaacaagtatagtgtgcggccaagccaagggaccatgccaccgtgctccaggcgttatgttgtcgtgacactgtcagcgcaagaggcggcgccgccatacatgcggtgtgacgacatgctcctagtgcagagcaccagcatcacccaagatcttggtgagatcaattatcaagaattgttcgacgtggccagggcggataaggtggttgatgtggtgcatctgccaatcgcatatgtcacgttagaagagtag

SEQ ID NO: 6 - protein, 2303 aa, Triticum aestivum
MRMGGTRALVRPWPACQRHKVKPLCGPFGAILPPQTLPHPARPTPFPVHGRRPAELLRAGRRPPPPRMAKKKKDKAPRKPRSECTPEEIAKLDAESVKRRGRRAVAKTNIAAAKRVAERAAIEAARHKAEVEEKEAIVSKARALLMAGICRPPGFSGRAVGPASTRSSVARPPHCQSPTSRTTPLSPGFPPPRHDGQTRFGGSPDVSMIAPSTPRPSAVIDLNVTLGSSSGGRPSVEMQRKQARLPFTGTMPSPRVLFDGMPTPTIPVDDPYQDGCGQFTADEEANDRADYDHGDSWHEDDDIYVEGDGDEEERNDVDISVEPLFIDELTQRAEAQKKRKSIRTSSYTQDEDKLICQAWMEISQDPRTGAQQKGIVFWTRVHKTFHERKLFEPYQFESNRGIGSIQKRWLFIQQECNKYQAAFESVQARPVSGLGVGDMAFQSLEAFKARHNDTPFTLTHCWTMINICPKFKDQYRELQRKRGLKTAKYAGGGDGEAFKRPRGKTNSKVDDIRDASSMALHDTLHDMMSQKDVRNEKKRQSNGKQMKQYLELQTKKLEMEEAAKRRKIGMEEEVRQRQLDIEAINAATKAKEVALAIMSVDLSKMSEKTRAWLAWVPRARWAAGHVPARKTFILKVGCVAGRWLCCRRGRPFILEAGCVSGRWRDGRVCRWLCCRHADMGLDARPPHLRPGPDTTPSPDQTDRIRTNRTSGSRGGVGLRPAVQARGAAQISTVGQEEKPEEPMKPEPDPGVAVWQPDGDGEIDMDLLPPISASLGAMASLSGKLDALQDTELKDEIRKLGSRLLKLSEPHEPRHAARIWMNEARELSYDMVNCVDADADWIDKMSRIFKPRVKEANGRYHRYKLESVPSRAAVLAIPMVVGDAGRKPDLLVGLHANGGAFETLRKNLIDRDEQLKALFVVGVGGIGKTTLAKELWREHKPGHHFCCRAFVRTAKKPDMRRILRSILAQVRPDQPPVANEVHELIHDLTEHLKDKRVGAAEACAAISLLTRGRRITTHGGWSSRPARRCGEGVDLRLSRPGPKPRRRSGCAAVAVRERHRRSIWVAREGEGAAAWGEEGGGRRRRRWERRYFIIIDDLWDTSVWDVAARAFPKGNQGSRIVTTTEIEDVALACCYQSKYVLKMEHLSESHSRELFTSAVFRSGEQHSHHVGEVPDEIIRRCAGLPQAIISISSVLASHGEANTVKNWEQIQNSLPTNTTSDEILKEVLIFCYNSLPSCVQTCLLHLSIYPENYVILKEDITKQWVAEGLISAPTEKEKMEIARSYFDMLVSMGMIQHIDVDYGNDVLYYAVHHMVHDIITSKSIEENFVKVIDYSQRAVRFSNKVSRLSLQFGGATYATTPARIELSQVRSLAYTGLKSCLPSISEFKLLRVLILHIWADQPSTCVTRKKKNQAQVTCNGTVHLPKQMRCLKHLETLEINATVAAIPSDIVHLRSLLHLRLGGGTELPDVTGVLTNVTLNLPSAATLLDDSSSSPDSLNTMELLPPICRIPNWIGQLTDLCILKVVVRELLRDDISNLERLPALTVLSLYVQQRNTELIIFEAGAFSALECFEFRCGELQLMFQEGAMPNLHRIKLGFNAHKGEQYDRLLSGIENLSDVQEISGIIGAAPGADEHDFQAAESAFMKAVSKLSSKVSVKRADMVEEEGGLAEKQDVIREKDASRHVISEQPAILKQESEEDIKQNAGGSLPSGIKNLSNVQEISGITGVATGAEEHEIQAAESALMKSVSEQPSKVTIKGADMVEQGYGPADKQHVSREKDVSSHLRSEQPAIVKQESGGNSQFIQWRSNSKETSNVVQGLSGNRELRGGAVGEVNKEEERQNSLARGKSSMDIKLVEIEAITNNFAEEQKVGSGGYGDVYRATHKGEEVAVKKLHQLQGLDDKQFDSEFRNLRNIRHQNVVRLIGYCHESRKKYMEHKGELIFAKEMERVLCFEYMHGGSLDKHITDESCELDWPTCYKIIKGTCEGLNHLHTSQGKPILHLDIKPANILLDKSMTPKIADLGLSKLVSSTLTHKTEIVKGTQGYMPPEYVDNGQISNKFDVFSFGVVIIKMMAGNVGYFRCAEMSHKEFIELVTKNWVKRLLTEPGYSSHETDMLGVTRCVEIALRCVDKDRNKRPCIKDVVHELEELEAEIKKMSLSSDQSKGLSLQASILRSCDTNILSVDPTLELRFVFEPRKETSCCLQMTNKTGGFIAFNILMNKNKYSVRPSQGTMPPCSRRYVVVTLSAQEAAPPYMRCDDMLLVQSTSITQDLGEINYQELFDVARADKVVDVVHLPIAYVTLEE

SEQ ID NO: 7 - DNA, 1173 bp, Artificial Sequence
  Probe LRR RGA 1
catggaatcatgaatcagttaatgttgtataagtccaggtcttcgaatttcatttctacatctattaatgataataaccgaagtaattaccgtcacctggttatccagaataacagaaacggtaaaagcttcagtccagaaacaagtgtcaagggcaagcagctgcgtccccggtctctaacagtctttgggagtgcagaagaagccgttccagatttgaagagttgtgagctgctgagagtgttggatctgaaagaatgcaatgatttgagggaccaacatctcgagcacatatacaagctgttgcatctaaaatatctggccctcggggattctagtagcaaatatctggatagaatgggaaagctacattgtttagagacactcgacttgaggaagaggaaaatcgagatactgccagtggaagtcatcagtttgccccacctagcacatctgttgggaaagttcaagctaaacaagttgggtaagaggaagcttaaagagttccggtcaaacaaatgcaacttggagactgtagcaggagttattgttgacagcgactctggattcctggaattgatggttcatttgaagcaacttagaaaggtcaagatatggtgcgagctcactagcacagattgcaagaacatactgggttcactttcaaaggccattcaaaagtttgctaaggatggcatagatactccagtaggtgaccgtggtcgcctatcactccatttcaacaattattctgaaggtctgttgcactgtgaagatgaccccacatttcttggttatcttaactcgctgaaactgcaaggcagcctgagtcagttccctaagtttgctaagtccctcgatggtctgcaagaactgtgccttacatatactaatctgacgggggctgatcttctactaggtctgtgtaggctacgacgcttggtttatctcaaactgatcgaagtccatcttgcggatttagacttagaagatggggatctcccaaaactgcaacgtctatgcctcgtggtgcaacagcccagattccccagtatccgaacaggcgctctgccgaaactaacttcaattcagttgctctgtggtggtctggaagatcttggtggcatcgaaatggaattgttcaaggacctccgggaaatcgctcttgattct

SEQ ID NO: 8 - DNA, 968 bp, Artificial Sequence
  Probe LRR RGA 2
gtgcatcacatggtacatgatatcattacatccaagtccatagaagagaattttgttaaagtaatagattattctcaaagggcggtacggttttctaacaaggttagtcgtctgtccctccagtttggcggtgcaacatatgcaactacaccagcacgtatcgaactgtcgcaagtgcgatctcttgcttatactggactgaagagctgcttgccttccatctcagagtttaagcttctccgggtactgattctccatatttgggctgatcaaccaagcacatgtgtcactcgcaaaaaaaagaaccaagcacaggtgtccacctcgagtgtatctctcgattgcttctattaatatatttgcaggtgacatgcaacggcaccgtgcatcttccaaaacagatgcgatgtctgaaacacttggaaacacttgaaataaatgcaacagtagcagccattccatcggatattgttcatcttcggagcttgttgcatctccgtctaggaggtgggacagaactgcctgatgtgacaggtgtcctcacaaatgttaccctgaatcttcctagtgctgccactttattggatgattcgagcagttctcccgattcactgaacacaatggagctattgccacccatttgcagaatccccaactggattggacagcttactgacctctgcattctgaaagttgtcgtcagagaactgctaagggatgatatcagtaacctggaaagattgccagcactcactgttctctccttgtacgtccagcaaagaaatacagaactaatcattttcgaagccggagcattttctgctctcgagtgttttgagttcaggtgtggtgaactgcagctgatgtttcaggaaggagcaatgcccaatcttcacagaatcaagctaggtttcaatgctcacaaaggagaacagtatgatcgtcttcttagcggcattgagaacctg

SEQ ID NO: 9 - DNA, 92 bp, Artificial Sequence
  Marker Wa_c6957_32R
cgggacagccaagagaaattccatttggcgatcgttcaaatgtgcactgcattctcgtactgccgtcgccgtcgtctgtctcttgactgtcg

SEQ ID NO: 10 - DNA, 92 bp, Artificial Sequence
  Marker Wa_c6957_32S
cgggacagccaagagaaattccatttggcgaccgttcaaatgtgcactgcattctcgtactgccgtcgccgtcgtctgtctcttgactgtcg

SEQ ID NO: 11 - DNA, 215 bp, Artificial Sequence
  Marker Excalibur_c1787R
catattgatgaacaagaacaagtatagtgtgcggccaagccaagggaccatgccaccgtgctccaggcgttatgttgtcgtgacgctgtcagcgcaagaggcggcgccgccatacatgcggtgtgacgacatgctcctagtgcagagcaccagcatcacccaagatcttggtgagatcaattatcaagaattgttcgacgtggccagggcggata

SEQ ID NO: 12 - DNA, 215 bp, Artificial Sequence
  Marker Excalibur_c1787_1301S
catattgatgaacaagaacaagtatagtgtgcggccaagccaagggaccatgccaccgtgctccaggcgttatgttgtcgtgacactgtcagcgcaagaggcggcgccgccatacatgcggtgtgacgacatgctcctagtgcagagcaccagcatcacccaagatcttggtgagatcaattatcaagaattgttcgacgtggccagggcggata

SEQ ID NO: 13 - DNA, 94 bp, Artificial Sequence
  Marker 1R
gtatgaaaagtatgaaaatagcacttgcttgtatgtagacctacggttttctaactatagacttagtaaacataccacatgaaataacatacca

SEQ ID NO: 14 - DNA, 96 bp, Artificial Sequence
  Marker 1S
tatcaaaagtatgaaaatagcacttgcttgtatgtagacctacggtttactaactatagacttagtaataaacataccacatgaaataacatacca

SEQ ID NO: 15 - DNA, 176 bp, Artificial Sequence
  Marker 2R
tgctcaacagctcaagtaccttttatcctttagatgctcggtgaggtcgtgaatgagctcgtgcacctcattagcgacgggtggttgatccggacgaacttgtgcgagtatgctcctcaggatcctcctcatgtcaggtttcttggcggtccgcacgaaagcccggcagcagaagt

SEQ ID NO: 16 - DNA, 160 bp, Artificial Sequence
  Marker 2S
taccttttatccttcagatgctcggtgaggtcatgaatgaggtcgtgcacctcattagcgtcgggtggttggtgcggacgaacttgtgcgagtatgctcctcaggatcctcctcatgtcaggtttcttggccgtccgcacaaaagctcggcagtcgaagt

SEQ ID NO: 17 - DNA, 176 bp, Artificial Sequence; identical to SEQ ID NO: 15
  Marker 3R

SEQ ID NO: 18 - DNA, 160 bp, Artificial Sequence; identical to SEQ ID NO: 16
  Marker 3S

SEQ ID NO: 19 - DNA, 176 bp, Artificial Sequence; identical to SEQ ID NO: 15
  Marker 4R

SEQ ID NO: 20 - DNA, 160 bp, Artificial Sequence; identical to SEQ ID NO: 16
  Marker 4S

SEQ ID NO: 21 - DNA, 144 bp, Artificial Sequence
  Marker 5R
ccaagtgttagtatactctaggaagctttatgcgccaactttgcatgtaggtaactaaaaactgggtgaaaaggttgctgacagagcctggatattcctcgcacgaaaccgacatgctaggagtcactagatgtgttgaaattg

SEQ ID NO: 22 - DNA, 144 bp, Artificial Sequence
  Marker 5S
ccaagtgttagtatactctaggaagctttatgcgccaactttgcatgtaggtaactaaaaactgggcgaaaaggttgctgacagagcctggatattcctcgcacgaaaccgacatgctaggagtcactagatgtgttgaaattg

SEQ ID NO: 23 - DNA, 16 bp, Artificial Sequence
  NBS1 8000 Primer F
cgacggcgcacgtgat

SEQ ID NO: 24 - DNA, 20 bp, Artificial Sequence
  NBS1 8000 Primer R
aacggacgacgaatgcaaat

SEQ ID NO: 25 - DNA, 16 bp, Artificial Sequence
  NBS1 8000 Probe MGB
tggactcgatccattg

SEQ ID NO: 26 - DNA, 55 bp, Artificial Sequence
  NBS1 8000 Amplicon or marker sequence
cgacggcgcacgtgatgctggactcgatccattgcatttgcattcgtcgtccgtt

SEQ ID NO: 27 - DNA, 19 bp, Artificial Sequence
  NBS4 4000 Primer F
acgctccgcaaaaatctga

SEQ ID NO: 28 - DNA, 21 bp, Artificial Sequence
  NBS4 4000 Primer R
aacaacgaatagcgccttgag

SEQ ID NO: 29 - DNA, 15 bp, Artificial Sequence
  NBS4 4000 Probe MGB
tgaccgggacgagca

SEQ ID NO: 30 - DNA, 57 bp, Artificial Sequence
  NBS4 4000 Amplicon or marker sequence
acgctccgcaaaaatctgattgaccgggacgagcagctcaaggcgctattcgttgtt

SEQ ID NO: 31 - DNA, 3000 bp, Triticum aestivum
gtcctacggactaaactctccggtttatatagacatcggaggaggctagtgagggagtcctggattagggggtatccggacagccggactgtatacatcttccggtctattgaagcgtgaagatacaagactcaagacttcggcccgtgtccggatgggactctcctttgtgtggaagacaagcttggcgatccggatattatatttccttccttgtaaccgactccatgtaaaccttagccctctccggtgtctatataaaccggagaggatggttcttagaaggccgatcacagttacaatcataccatcataggctagctcctagggtttagcctctacgatctcgtggtagatcaactcttgtactacacatatcttcaatattaatcaagcatgaagtagggttttacctcaatcgagagggctcgaacctgagtaaacattgtgtcccttgcttactgttaccatcagcctaagacgcacaaatcgggaccccctacccgagatccgccggttttgacaccgacattggtgctttcattgagagtttctctgtgtcgtcgctttgaggcttgatggcgtcttcaatcgccaacaacaccgtccagggcgagacttttctccccggacagatctttgtgttcggcggcttcgcactgcgggccaattcgcttggtcatctggagcagatcgacagctacgcccctggccaccagatcaggttcggaaacttgaactacacggcggatatttgcggagacttgatcttcgacggattcggccctgtgccaggagcgccggacaatcacgacgagcacggcctagacctgttgtcggacaattctcagaacatcatccctgaaatagccccggatctaaatccggaacaggttgtgttgcccaaggacggagggatagaccccgtcccgcaggccacatactcatcggcggtggagccgaacacaggtctcacctctgtggaagccagtaaccccggccccccggactcatatccggttgttggttccggtctgcacacccccgagccagtcgaaccaggctaggctccggtaatggagcttaccgctgcggacatctttcaacactcgccctttggcgacatgttgaattcattaaagtctctctctttgttaggaggctctgggccgaactatgtccggcctgagtgggaagcaggcgacgaaggaattcgttgcccacccagcacccacttcattgccacggtcgacgatttaaccgacgtgcttaactttgactccaaagatatcgacggtatggacgacgatgcaggagacgtacaggagccaccgctcatagggcggtggacggccacctcctcatacgatatatacacggtggacactccgaaggaaaccaatggcgacgaggcagcggaggataacccctcgggaggaaaagcaaaacatgggcgtcttcggcgtcgctccaagccccgccacatcaataccgtccccggagatgatccggacagtgccgaagaggaatacagccctgatcaggccaccttcaagcaggccggacaggccacgttgggatacttggaaagggacaactatacagccccctccaaagatgaggtaagcctcagcaatgacgaattcggtgtgcctgaagatccagtggaacagttcgcttcaagcgacggctcatggccacggcaaggtgcctgcacaggaagcaagagcagcttaaagccaaccaggatttgctaatggacaggtggaccaagatcctggccaccgaaaagtacggactcgaccaccccagcaaagggcatacgcggcacaactggctacctcaacctaagcaggagaaccaaaagcacacaacccgacgtccgcacaccactacggtccaagacagcaagaagaatacatgaagaggcatcctcaagcctcggcgcaatggtcataaacgtcaagtcagggacgctggtgccaagtccagcaactcccagtctgatcaacggacaaagagcagctcaagcctattcggcccaagccacaaactcgatcaaccgtgtgaaattaacggtactcccagaaggacggcaaaacataccaatagagaatgccggatcttcaaacaaagcgaccggtcgtgtgccggaaacaatgaagggaggcgtctagtcaagagacccccccccagagcacaacagtacggccgatcgcccctaccatacaaaccacagcaattaaattttcgtacccccagacccagtagtccaggggctccataacacataaagcctccgcgggtatgaatctacaaataacaccttctacaaaatgtcaggtgcaaaggccaagttcattggcccaccgctctaacggttgctttcagataaccaaaaaatgtcacgtcatcggtgcattcccctcatacggtaacccaccgtctgctaacgggatgaaccacgttgactagattccacgtggtaaaccattaggccaacaccagtgatatactcacgcctacgtacaaggccgaacccctcccctagagcggaaatcatacagctgccggagtagcaagtcatgcatgcctatcaatattttgatatgacatccaactattcggacaccaactgaggagtccgcgctgcttctcggtatatcggctagggtcaccagggtccgatcaggaacctttagcccaactgtcggtgtcaaaaccggcggatctcgggtagagggtcccgaactgtgcgtctaggcggatggtaacaggagacaagggacacgatgtttttacccaggttcgggccctctcgatggaggtaaaaccctactcctgcttgattaatattgatgatatggatagtacaagagtagatctaccacgagatcagagaggctaaaccctagaagctagcctatgttatgattgttgtttgtcctacggactaaaaccctccggtttatataggcaccgaatagggttagggttaca

SEQ ID NO: 32 - DNA, 3000 bp, Triticum aestivum
tcttttcatttaattttatatcctttagcagtagcgagtttagattaaaacgcgctgctacaaataaagtaccggtagcgcggttcgttataggtcgctactactatgtgtagcctatcggctaagccgtgggaattttagtagtaacgtgtttagagcaagacgcgctactgctagaactttatctgcagcgcggtttgctcaggcgcgctactgctacttagcaccagcgtgcttttttgaccctcgctactgctaaagttctgtgtataaggttttccctagtagtgttactacggaagaccatagctctcactttccataaaagtgttctatctaaaacgtttatgatgaatagctgcacaaatcctgctcggcacattttcccttggcttactggggaagctgtcggtttatatacggatgttctatctaaaacgtttgcgatcaagagctgcacaactcgtcacattttcgctaggcttcccggggaagctgttggtttgcatacgggtgttctaactaaaacttttgcaatgagtgttttatatttaaaaattgtattaaactgcggcatgggcgccattaatgtagaggatgcgagcaaggcggccggccatggaagtcaaagggctcacttcccagtgagcttgcgcggcatacagctcacacgctttccggtgagcctgcacattggagtacagctcgcacacctcccgtttagtcaagcacctgtttgcatgacacctcctagccattaaaagagtgaggcgtgacatcacgtgaatggttaagataacacacacgttttaaattatttaaaatgtttgagatgttacagtggcagcaatttgtttcaaaatgcctttgttggctgttatttgagtgcgccttctctcaaaatggacacaaaaaataccacaacatgtcgggtgccatttcatgatagcatgccaagtttcatgaattttcgacgagttttggatttactagaatttaaaaacagagtatttcaacattttgtcggcaatcaatagtgccctggtgtttgaaattcattctaatttcttgcatgagacttaagcatgcacccaaggacacatatttgattttccaaccaatttatatgcactggagcatgtgcatgtagttcaaatttgaattatgcacataaaatgcctagaaaacccagttaatgtataaaaatgaccaaacgagccctatttttttttcaaaatttaacacaacactcctgttattctatgttgacactagaaattttttgaaagcaataagaggcaacggatatcattttgtccctaaagtggcacgttccctaccgaagacatcaggcttgttgtgagaagctccggtttgtgagaagcttatacccaaacctgccccaaatgggacaaaaattttaccacggcatgttgatgccgctccatgatagtatgcgaagtttcatgaatttcagacaagttatggatttactaaaatttaaaaaccatgtatctcaatgtttgcggccgagtgacgatggcagggtgtttgacatccattcccatttcttgcatgggacctaagcatgcaaccaatgacacatatttgaattttcaaccaatttatatgcactaaagcatgtgcctgtagttcaaatttgtgagaacgttaacgtcattgtgagaacccgacattccaaaaaaagcatgccaaatctataagtcatgtgatgccgctgcttctatagtatgatggtggcctctttgatgtgccctcgatacattctccgcaaagccttgtggcagttcttccattgccaatgcatgcaatcaattgatgcgagcatccatggaaattctcaggcctctcaagtagccaacaactcctctctgtcgtgtgcatttggttctctcagatactctgctccaaacacctgcaccatggcacgggcaaacttgacagtagtcttcaggcatgcgctctcccccatactgacaatctcaccaatgagagtacctagtgtaagcatcctcagagcagctgcgcacttctgtttagcagagaaagaaagttggctgcaacaatccctcgtgagcttgaagtagtcatcatgtgccttcattccctccattatgcgcaaaacaatggttttcgcatgcgaaaaccgcgaagaaaccatggatcatctaggaaagttggatttcgagcaaagtagtccttctgtagtaggcatgctccggactccctgcccgattgaccactcttctccctttgattgagtccttgaagttgagaatatgctccacttgccggtccatttcttcttgcatgctcatcggcatgatcatgtccacttcttctccgaatacgaggaatcgaagaactcatcttgaaccatttgatcaagcttcgtcggtccatactcggtgtgcgacgaagcatcaggatccattgttttctctataaaaatcacaaaaaaaactaggttgaggaatgtgtcgaacacatagagtgtaaggggtgcctgggagttgccagacgtaccgcggtggcgtccggactggcgatgacatccccgtcagcgaggatagaagggaggagtgttgtgccagttctggaggcgcagaggctctaaacagcggtggatctgcgagacggacatcgtgaaggaggaagaagagataagagaccaaatgaatccggtaggtcaaggggatggatttggtgcaatttgagttaggataaagctgtcgggtctgacatggcagatgcgcctggacgcgcccatatctgccccatatttgggcaacatatgaggggtgtcggtcagtcggggcggttgagaccgtttgaggtgcccgtctgagtcggattttggtgaccgatcaataaccatgccgttcgctcggtcgtttaaggtgggtttggaacgtccagctgcagatgctcttatatgaatttaggtgcgggaatatgacgagtactattattgcggac

SEQ ID NO: 33 - DNA, 2750 bp, Triticum aestivum
tgtctatataaaccggagaggatggttcttagaaggccgatcacagttacaatcataccatcataggctagctcctagggtttagcctctacgatctcgtggtagatcaactcttgtactacacatatcttcaatattaatcaagcatgaagtagggttttacctcaatcgagagggctcgaacctgagtaaacattgtgtcccttgcttactgttaccatcagcctaagacgcacaaatcgggaccccctacccgagatccgccggttttgacaccgacattggtgctttcattgagagtttctctgtgtcgtcgctttgaggcttgatggcgtcttcaatcgccaacaacaccgtccagggcgagacttttctccccggacagatctttgtgttcggcggcttcgcactgcgggccaattcgcttggtcatctggagcagatcgacagctacgcccctggccaccagatcaggttcggaaacttgaactacacggcggatatttgcggagacttgatcttcgacggattcggccctgtgccaggagcgccggacaatcacgacgagcacggcctagacctgttgtcggacaattctcagaacatcatccctgaaatagccccggatctaaatccggaacaggttgtgttgcccaaggacggagggatagaccccgtcccgcaggccacatactcatcggcggtggagccgaacacaggtctcacctctgtggaagccagtaaccccggccccccggactcatatccggttgttggttccggtctgcacacccccgagccagtcgaaccaggctaggctccggtaatggagcttaccgctgcggacatctttcaacactcgccctttggcgacatgttgaattcattaaagtctctctctttgttaggaggctctgggccgaactatgtccggcctgagtgggaagcaggcgacgaaggaattcgttgcccacccagcacccacttcattgccacggtcgacgatttaaccgacgtgcttaactttgactccaaagatatcgacggtatggacgacgatgcaggagacgtacaggagccaccgctcatagggcggtggacggccacctcctcatacgatatatacacggtggacactccgaaggaaaccaatggcgacgaggcagcggaggataacccctcgggaggaaaagcaaaacatgggcgtcttcggcgtcgctccaagccccgccacatcaataccgtccccggagatgatccggacagtgccgaagaggaatacagccctgatcaggccaccttcaagcaggccggacaggccacgttgggatacttggaaagggacaactatacagccccctccaaagatgaggtaagcctcagcaatgacgaattcggtgtgcctgaagatccagtggaacagttcgcttcaagcgacggctcatggccacggcaaggtgcctgcacaggaagcaagagcagcttaaagccaaccaggatttgctaatggacaggtggaccaagatcctggccaccgaaaagtacggactcgaccaccccagcaaagggcatacgcggcacaactggctacctcaacctaagcaggagaaccaaaagcacacaacccgacgtccgcacaccactacggtccaagacagcaagaagaatacatgaagaggcatcctcaagcctcggcgcaatggtcataaacgtcaagtcagggacgctggtgccaagtccagcaactcccagtctgatcaacggacaaagagcagctcaagcctattcggcccaagccacaaactcgatcaaccgtgtgaaattaacggtactcccagaaggacggcaaaacataccaatagagaatgccggatcttcaaacaaagcgaccggtcgtgtgccggaaacaatgaagggaggcgtctagtcaagagacccccccccagagcacaacagtacggccgatcgcccctaccatacaaaccacagcaattaaattttcgtacccccagacccagtagtccaggggctccataacacataaagcctccgcgggtatgaatctacaaataacaccttctacaaaatgtcaggtgcaaaggccaagttcattggcccaccgctctaacggttgctttcagataaccaaaaaatgtcacgtcatcggtgcattcccctcatacggtaacccaccgtctgctaacgggatgaaccacgttgactagattccacgtggtaaaccattaggccaacaccagtgatatactcacgcctacgtacaaggccgaacccctcccctagagcggaaatcatacagctgccggagtagcaagtcatgcatgcctatcaatattttgatatgacatccaactattcggacaccaactgaggagtccgcgctgcttctcggtatatcggctagggtcaccagggtccgatcaggaacctttagcccaactgtcggtgtcaaaaccggcggatctcgggtagagggtcccgaactgtgcgtctaggcggatggtaacaggagacaagggacacgatgtttttacccaggttcgggccctctcgatggaggtaaaaccctactcctgcttgattaatattgatgatatggatagtacaagagtagatctaccacgagatcagagaggctaaaccctagaagctagcctatgttatgattgttgtttgtcctacggactaaaaccctccggtttatataggcaccgaatagggttagggttaca

SEQ ID NO: 34 - DNA, 1637 bp, Triticum aestivum
atacgatatatacacggtggacactccgaaggaaaccaatggcgacgaggcagcggaggataacccctcgggaggaaaagcaaaacatgggcgtcttcggcgtcgctccaagccccgccacatcaataccgtccccggagatgatccggacagtgccgaagaggaatacagccctgatcaggccaccttcaagcaggccggacaggccacgttgggatacttggaaagggacaactatacagccccctccaaagatgaggtaagcctcagcaatgacgaattcggtgtgcctgaagatccagtggaacagttcgcttcaagcgacggctcatggccacggcaaggtgcctgcacaggaagcaagagcagcttaaagccaaccaggatttgctaatggacaggtggaccaagatcctggccaccgaaaagtacggactcgaccaccccagcaaagggcatacgcggcacaactggctacctcaacctaagcaggagaaccaaaagcacacaacccgacgtccgcacaccactacggtccaagacagcaagaagaatacatgaagaggcatcctcaagcctcggcgcaatggtcataaacgtcaagtcagggacgctggtgccaagtccagcaactcccagtctgatcaacggacaaagagcagctcaagcctattcggcccaagccacaaactcgatcaaccgtgtgaaattaacggtactcccagaaggacggcaaaacataccaatagagaatgccggatcttcaaacaaagcgaccggtcgtgtgccggaaacaatgaagggaggcgtctagtcaagagacccccccccagagcacaacagtacggccgatcgcccctaccatacaaaccacagcaattaaattttcgtacccccagacccagtagtccaggggctccataacacataaagcctccgcgggtatgaatctacaaataacaccttctacaaaatgtcaggtgcaaaggccaagttcattggcccaccgctctaacggttgctttcagataaccaaaaaatgtcacgtcatcggtgcattcccctcatacggtaacccaccgtctgctaacgggatgaaccacgttgactagattccacgtggtaaaccattaggccaacaccagtgatatactcacgcctacgtacaaggccgaacccctcccctagagcggaaatcatacagctgccggagtagcaagtcatgcatgcctatcaatattttgatatgacatccaactattcggacaccaactgaggagtccgcgctgcttctcggtatatcggctagggtcaccagggtccgatcaggaacctttagcccaactgtcggtgtcaaaaccggcggatctcgggtagagggtcccgaactgtgcgtctaggcggatggtaacaggagacaagggacacgatgtttttacccaggttcgggccctctcgatggaggtaaaaccctactcctgcttgattaatattgatgatatggatagtacaagagtagatctaccacgagatcagagaggctaaaccctagaagctagcctatgttatgattgttgtttgtcctacggactaaaaccctccggtttatataggcaccgaatagggttagggttaca

SEQ ID NO: 35 - DNA, 410 bp, Triticum aestivum
tgcctatcaatattttgatatgacatccaactattcggacaccaactgaggagtccgcgctgcttctcggtatatcggctagggtcaccagggtccgatcaggaacctttagcccaactgtcggtgtcaaaaccggcggatctcgggtagagggtcccgaactgtgcgtctaggcggatggtaacaggagacaagggacacgatgtttttacccaggttcgggccctctcgatggaggtaaaaccctactcctgcttgattaatattgatgatatggatagtacaagagtagatctaccacgagatcagagaggctaaaccctagaagctagcctatgttatgattgttgtttgtcctacggactaaaaccctccggtttatataggcaccgaatagggttagggttaca

SEQ ID NO: 36 - DNA, 2094 bp, Triticum aestivum
acacaaaaaataccacaacatgtcgggtgccatttcatgatagcatgccaagtttcatgaattttcgacgagttttggatttactagaatttaaaaacagagtatttcaacattttgtcggcaatcaatagtgccctggtgtttgaaattcattctaatttcttgcatgagacttaagcatgcacccaaggacacatatttgattttccaaccaatttatatgcactggagcatgtgcatgtagttcaaatttgaattatgcacataaaatgcctagaaaacccagttaatgtataaaaatgaccaaacgagccctatttttttttcaaaatttaacacaacactcctgttattctatgttgacactagaaattttttgaaagcaataagaggcaacggatatcattttgtccctaaagtggcacgttccctaccgaagacatcaggcttgttgtgagaagctccggtttgtgagaagcttatacccaaacctgccccaaatgggacaaaaattttaccacggcatgttgatgccgctccatgatagtatgcgaagtttcatgaatttcagacaagttatggatttactaaaatttaaaaaccatgtatctcaatgtttgcggccgagtgacgatggcagggtgtttgacatccattcccatttcttgcatgggacctaagcatgcaaccaatgacacatatttgaattttcaaccaatttatatgcactaaagcatgtgcctgtagttcaaatttgtgagaacgttaacgtcattgtgagaacccgacattccaaaaaaagcatgccaaatctataagtcatgtgatgccgctgcttctatagtatgatggtggcctctttgatgtgccctcgatacattctccgcaaagccttgtggcagttcttccattgccaatgcatgcaatcaattgatgcgagcatccatggaaattctcaggcctctcaagtagccaacaactcctctctgtcgtgtgcatttggttctctcagatactctgctccaaacacctgcaccatggcacgggcaaacttgacagtagtcttcaggcatgcgctctcccccatactgacaatctcaccaatgagagtacctagtgtaagcatcctcagagcagctgcgcacttctgtttagcagagaaagaaagttggctgcaacaatccctcgtgagcttgaagtagtcatcatgtgccttcattccctccattatgcgcaaaacaatggttttcgcatgcgaaaaccgcgaagaaaccatggatcatctaggaaagttggatttcgagcaaagtagtccttctgtagtaggcatgctccggactccctgcccgattgaccactcttctccctttgattgagtccttgaagttgagaatatgctccacttgccggtccatttcttcttgcatgctcatcggcatgatcatgtccacttcttctccgaatacgaggaatcgaagaactcatcttgaaccatttgatcaagcttcgtcggtccatactcggtgtgcgacgaagcatcaggatccattgttttctctataaaaatcacaaaaaaaactaggttgaggaatgtgtcgaacacatagagtgtaaggggtgcctgggagttgccagacgtaccgcggtggcgtccggactggcgatgacatccccgtcagcgaggatagaagggaggagtgttgtgccagttctggaggcgcagaggctctaaacagcggtggatctgcgagacggacatcgtgaaggaggaagaagagataagagaccaaatgaatccggtaggtcaaggggatggatttggtgcaatttgagttaggataaagctgtcgggtctgacatggcagatgcgcctggacgcgcccatatctgccccatatttgggcaacatatgaggggtgtcggtcagtcggggcggttgagaccgtttgaggtgcccgtctgagtcggattttggtgaccgatcaataaccatgccgttcgctcggtcgtttaaggtgggtttggaacgtccagctgcagatgctcttatatgaatttaggtgcgggaatatgacgagtactattattgcggac

SEQ ID NO: 37 - DNA, 540 bp, Triticum aestivum
tctctataaaaatcacaaaaaaaactaggttgaggaatgtgtcgaacacatagagtgtaaggggtgcctgggagttgccagacgtaccgcggtggcgtccggactggcgatgacatccccgtcagcgaggatagaagggaggagtgttgtgccagttctggaggcgcagaggctctaaacagcggtggatctgcgagacggacatcgtgaaggaggaagaagagataagagaccaaatgaatccggtaggtcaaggggatggatttggtgcaatttgagttaggataaagctgtcgggtctgacatggcagatgcgcctggacgcgcccatatctgccccatatttgggcaacatatgaggggtgtcggtcagtcggggcggttgagaccgtttgaggtgcccgtctgagtcggattttggtgaccgatcaataaccatgccgttcgctcggtcgtttaaggtgggtttggaacgtccagctgcagatgctcttatatgaatttaggtgcgggaatatgacgagtactattattgcggac